European Patent Application EP 4 763 982 A2, published June 24, 2026. Title: ONCOLYTIC VIRUS THERAPY. Applicant: University of Pittsburgh - Of the Commonwealth System of Higher Education. Application EP not yet assigned, filed February 5, 2018. The sequence listing filed with the application follows.

SEQUENCE LISTING (36 sequences)

SEQ ID NO: 1 - protein, 34 aa, Homo sapiens
SSFSPPGYQVSFCLVMVLLFAVDTGLYFSVKTNI

SEQ ID NO: 2 - protein, 22 aa, Homo sapiens
GGALQSTASLFVVSLSLLHLYS

SEQ ID NO: 3 - protein, 24 aa, Homo sapiens
NNSCSSPGGCRLFLSTIPVLWTLL

SEQ ID NO: 4 - protein, 28 aa, Homo sapiens
DAAHPGRSVVPALLPLLAGTLLLLETAT

SEQ ID NO: 5 - protein, 23 aa, Homo sapiens
SAAPRLFPLAWTVLLLPLLLLQT

SEQ ID NO: 6 - protein, 24 aa, Homo sapiens
NGSISLAVPLWLLAASLLCLLSCK

SEQ ID NO: 7 - protein, 26 aa, Homo sapiens
SGAPTLSPSLLGLLLPAFGILVYLEF

SEQ ID NO: 8 - protein, 24 aa, Rattus sp.
NGTSRRAGCIWLLPLLVLHLLLKF

SEQ ID NO: 9 - protein, 29 aa, synthetic construct
  REGION 1..29: note = Description of Artificial Sequence: Synthetic peptide
NSTGSGSSGSAAAAVAAAAVAAAAVAAAA

SEQ ID NO: 10 - protein, 29 aa, synthetic construct
  REGION 1..29: note = Description of Artificial Sequence: Synthetic peptide
NSTGSGSSGSAAAAVVFVFVFVFVVAAAA

SEQ ID NO: 11 - protein, 38 aa, Homo sapiens
VSTISSFSPPGYQVSFCLVMVLLFAVDTGLYFSVKTNI

SEQ ID NO: 12 - protein, 15 aa, synthetic construct
  REGION 1..15: note = Description of Artificial Sequence: Synthetic peptide
GGGGSGGGGSGGGGS

SEQ ID NO: 13 - protein, 133 aa, Homo sapiens [sequence omitted]

SEQ ID NO: 14 - protein, 189 aa, synthetic construct
  REGION 1..189: note = Description of Artificial Sequence: Synthetic polypeptide
APTSSSTKKTQLQLEHLLLDLQMILNGINNYKNPKLTRMLTFKFYMPKKATELKHLQCLEEELKPLEEVLNLAQSKNFHLRPRDLISNINVIVLELKGSETTFMCEYADETATIVEFLNRWITFCQSIISTLTGPAGGGGSGGGGSGGGGSVSTISSFSPPGYQVSFCLVMVLLFAVDTGLYFSVKTNI

SEQ ID NO: 15 - protein, 233 aa, Homo sapiens
MSTESMIRDVELAEEALPKKTGGPQGSRRCLFLSLFSFLIVAGATTLFCLLHFGVIGPQREEFPRDLSLISPLAQAVRSSSRTPSDKPVAHVVANPQAEGQLQWLNRRANALLANGVELRDNQLVVPSEGLYLIYSQVLFKGQGCPSTHVLLTHTISRIAVSYQTKVNLLSAIKSPCQRETPEGAEAKPWYEPIYLGGVFQLEKGDRLSAEINRPDYLDFAESGQVYFGIIAL

SEQ ID NO: 16 - protein, 56 aa, synthetic construct
  REGION 1..56: note = Description of Artificial Sequence: Synthetic polypeptide
GPAGGGGSGGGGSGGGGSVSTISSFSPPGYQVSFCLVMVLLFAVDTGLYFSVKTNI

SEQ ID NO: 17 - protein, 10 aa, synthetic construct
  REGION 1..10: note = Description of Artificial Sequence: Synthetic peptide
NSTGSGSSGS

SEQ ID NO: 18 - protein, 189 aa, Homo sapiens
MLGSRAVMLLLLLPWTAQGRAVPGGSSPAWTQCQQLSQKLCTLAWSAHPLVGHMDLREEGDEETTNDVPHIQCGDGCDPQGLRDNSQFCLQRIHQGLIFYEKLLGSDIFTGEPSLLPDSPVGQLHASLLGLSQLLQPEGHHWETQQIPSLSPSQPWQRLLLRFKILRSLQAFVAVAARVFAHGAATLSP

SEQ ID NO: 19 - DNA, 55 bp, synthetic construct
  misc_feature 1..55: note = Description of Artificial Sequence: Synthetic primer
  source 1..55: mol_type = other DNA
gcgggtcgacatatggcgccatgcattataaggcgcgcccgcccctctccctccc

SEQ ID NO: 20 - DNA, 55 bp, synthetic construct
  misc_feature 1..55: note = Description of Artificial Sequence: Synthetic primer
  source 1..55: mol_type = other DNA
ggccgttaacttaagagctcatttaaatcctgcagggccggccattatcatcgtg

SEQ ID NO: 21 - DNA, 54 bp, synthetic construct
  misc_feature 1..54: note = Description of Artificial Sequence: Synthetic primer
  source 1..54: mol_type = other DNA
ggccggccggccggtggcggtgggagcggtggtgggggttccggaggcggaggg

SEQ ID NO: 22 - DNA, 44 bp, synthetic construct
  misc_feature 1..44: note = Description of Artificial Sequence: Synthetic primer
  source 1..44: mol_type = other DNA
ggttccggaggcggagggtcggtgtcaaccatctcatcattctc

SEQ ID NO: 23 - DNA, 32 bp, synthetic construct
  misc_feature 1..32: note = Description of Artificial Sequence: Synthetic primer
  source 1..32: mol_type = other DNA
gcgcgttaactcaaatgtttgtcttcacagag

SEQ ID NO: 24 - DNA, 60 bp, synthetic construct
  misc_feature 1..60: note = Description of Artificial Sequence: Synthetic primer
  source 1..60: mol_type = other DNA
ggccggccggccgctgaagctgccgcaaaagaggccgctgcgaaggaggccgcggctaag

SEQ ID NO: 25 - DNA, 60 bp, synthetic construct
  misc_feature 1..60: note = Description of Artificial Sequence: Synthetic primer
  source 1..60: mol_type = other DNA
gaggccgcggctaaggaggcggcagctaaagctgcagccgtgtcaaccatctcatcattc

SEQ ID NO: 26 - DNA, 32 bp, synthetic construct; identical to SEQ ID NO: 23
  misc_feature 1..32: note = Description of Artificial Sequence: Synthetic primer
  source 1..32: mol_type = other DNA

SEQ ID NO: 27 - DNA, 29 bp, synthetic construct
  misc_feature 1..29: note = Description of Artificial Sequence: Synthetic primer
  source 1..29: mol_type = other DNA
ggcggtcgacatgtacagcatgcagctcg

SEQ ID NO: 28 - DNA, 31 bp, synthetic construct
  misc_feature 1..31: note = Description of Artificial Sequence: Synthetic primer
  source 1..31: mol_type = other DNA
ccgcggcgcgccttattgagggcttgttgag

SEQ ID NO: 29 - DNA, 29 bp, synthetic construct
  misc_feature 1..29: note = Description of Artificial Sequence: Synthetic primer
  source 1..29: mol_type = other DNA
ggcggtcgacatgtacagcatgcagctcg

SEQ ID NO: 30 - DNA, 29 bp, synthetic construct
  misc_feature 1..29: note = Description of Artificial Sequence: Synthetic primer
  source 1..29: mol_type = other DNA
ccgcggccggcccttgagggcttgttgag

SEQ ID NO: 31 - DNA, 29 bp, synthetic construct
  misc_feature 1..29: note = Description of Artificial Sequence: Synthetic primer
  source 1..29: mol_type = other DNA
ggcggtcgacatgtacagcatgcagctcg

SEQ ID NO: 32 - DNA, 29 bp, synthetic construct
  misc_feature 1..29: note = Description of Artificial Sequence: Synthetic primer
  source 1..29: mol_type = other DNA
ccgcggccggcccttgagggcttgttgag

SEQ ID NO: 33 - DNA, 54 bp, synthetic construct; identical to SEQ ID NO: 21
  misc_feature 1..54: note = Description of Artificial Sequence: Synthetic primer
  source 1..54: mol_type = other DNA

SEQ ID NO: 34 - DNA, 37 bp, synthetic construct
  misc_feature 1..37: note = Description of Artificial Sequence: Synthetic primer
  source 1..37: mol_type = other DNA
ccggaggcggtgggtcgcactgggtgcttctgggatc

SEQ ID NO: 35 - DNA, 60 bp, synthetic construct
  misc_feature 1..60: note = Description of Artificial Sequence: Synthetic primer
  source 1..60: mol_type = other DNA
cgcgttaactaccccaagaagaggaggaccgtggacactacaatgaggaacaacaggatg

SEQ ID NO: 36 - protein, 24 aa, synthetic construct
  REGION 1..24: note = Description of Artificial Sequence: Synthetic peptide
AEAAAKEAAAKEAAAKEAAAKAAA